European Patent Application EP 4 261 222 A1, published October 18, 2023. Title: Anti-OX40L antibody, anti-OX40L and anti-TNFa bispecific antibody, and uses thereof. Applicant: HK INNO.N CORPORATION Y-BIOLOGICS INC. The sequence listing filed with the application follows.

SEQUENCE LISTING (94 sequences)

SEQ ID NO: 1 - protein, 183 aa, Unknown
  OX40L seq
MERVQPLEENVGNAARPRFERNKLLLVASVIQGLGLLLCFTYICLHFSALQVSHRYPRIQSIKVQFTEYKKEKGFILTSQKEDEIMKVQNNSVIINCDGFYLISLKGYFSQEVNISLHYQKDEEPLFQLKKVRSVNSLMVASLTYKDKVYLNVTTDNTSLDDFHVNGGELILIHQNPGEFCVL

SEQ ID NO: 2 - protein, 139 aa, Artificial Sequence
  OX40L-his
HHHHHHQVSHRYPRIQSIKVQFTEYKKEKGFILTSQKEDEIMKVQNNSVIINCDGFYLISLKGYFSQEVNISLHYQKDEEPLFQLKKVRSVNSLMVASLTYKDKVYLNVTTDNTSLDDFHVNGGELILIHQNPGEFCVL

SEQ ID NO: 3 - protein, 8 aa, Artificial Sequence
  epitope 93-100
VIINCDGF

SEQ ID NO: 4 - protein, 11 aa, Artificial Sequence
  epitope 141-151
ASLTYKDKVYL

SEQ ID NO: 5 - protein, 330 aa, Artificial Sequence [sequence omitted]

SEQ ID NO: 6 - protein, 330 aa, Artificial Sequence
  IgG1 HC N297A
ASTKGPSVFPLAPSSKSTSGGTAALGCLVKDYFPEPVTVSWNSGALTSGVHTFPAVLQSSGLYSLSSVVTVPSSSLGTQTYICNVNHKPSNTKVDKKVEPKSCDKTHTCPPCPAPELLGGPSVFLFPPKPKDTLMISRTPEVTCVVVDVSHEDPEVKFNWYVDGVEVHNAKTKPREEQYASTYRVVSVLTVLHQDWLNGKEYKCKVSNKALPAPIEKTISKAKGQPREPQVYTLPPSRDELTKNQVSLTCLVKGFYPSDIAVEWESNGQPENNYKTTPPVLDSDGSFFLYSKLTVDKSRWQQGNVFSCSVMHEALHNHYTQKSLSLSPGK

SEQ ID NO: 7 - protein, 327 aa, Artificial Sequence
  IgG4 HC
ASTKGPSVFPLAPCSRSTSESTAALGCLVKDYFPEPVTVSWNSGALTSGVHTFPAVLQSSGLYSLSSVVTVPSSSLGTKTYTCNVDHKPSNTKVDKRVESKYGPPCPSCPAPEFLGGPSVFLFPPKPKDTLMISRTPEVTCVVVDVSQEDPEVQFNWYVDGVEVHNAKTKPREEQFNSTYRVVSVLTVLHQDWLNGKEYKCKVSNKGLPSSIEKTISKAKGQPREPQVYTLPPSQEEMTKNQVSLTCLVKGFYPSDIAVEWESNGQPENNYKTTPPVLDSDGSFFLYSRLTVDKSRWQEGNVFSCSVMHEALHNHYTQKSLSLSLGK

SEQ ID NO: 8 - protein, 327 aa, Artificial Sequence
  IgG4 HC S228P
ASTKGPSVFPLAPCSRSTSESTAALGCLVKDYFPEPVTVSWNSGALTSGVHTFPAVLQSSGLYSLSSVVTVPSSSLGTKTYTCNVDHKPSNTKVDKRVESKYGPPCPPCPAPEFLGGPSVFLFPPKPKDTLMISRTPEVTCVVVDVSQEDPEVQFNWYVDGVEVHNAKTKPREEQFNSTYRVVSVLTVLHQDWLNGKEYKCKVSNKGLPSSIEKTISKAKGQPREPQVYTLPPSQEEMTKNQVSLTCLVKGFYPSDIAVEWESNGQPENNYKTTPPVLDSDGSFFLYSRLTVDKSRWQEGNVFSCSVMHEALHNHYTQKSLSLSLGK

SEQ ID NO: 9 - DNA, 981 bp, Artificial Sequence
  IgG4 HC S228P
gcttccaccaagggcccatccgtcttccccctggcgccctgctccaggagcacctccgagagcacagccgccctgggctgcctggtcaaggactacttccccgaaccggtgacggtgtcgtggaactcaggcgccctgaccagcggcgtgcacaccttcccggctgtcctacagtcctcaggactctactccctcagcagcgtggtgaccgtgccctccagcagcttgggcacgaagacctacacctgcaacgtagatcacaagcccagcaacaccaaggtggacaagagagttgagtccaaatatggtcccccatgcccaccatgcccagcacctgagttcctggggggaccatcagtcttcctgttccccccaaaacccaaggacactctcatgatctcccggacccctgaggtcacgtgcgtggtggtggacgtgagccaggaagaccccgaggtccagttcaactggtacgtggatggcgtggaggtgcataatgccaagacaaagccgcgggaggagcagttcaacagcacgtaccgtgtggtcagcgtcctcaccgtcctgcaccaggactggctgaacggcaaggagtacaagtgcaaggtctccaacaaaggcctcccgtcctccatcgagaaaaccatctccaaagccaaagggcagccccgagagccacaggtgtacaccctgcccccatcccaggaggagatgaccaagaaccaggtcagcctgacctgcctggtcaaaggcttctaccccagcgacatcgccgtggagtgggagagcaatgggcagccggagaacaactacaagaccacgcctcccgtgctggactccgacggctccttcttcctctacagcaggctaaccgtggacaagagcaggtggcaggaggggaatgtcttctcatgctccgtgatgcatgaggctctgcacaaccactacacacagaagagcctctccctgtctctgggtaaa

SEQ ID NO: 10 - protein, 107 aa, Artificial Sequence [sequence omitted]

SEQ ID NO: 11 - DNA, 321 bp, Artificial Sequence
  IgG LC
cgtacggtggcggcgccatctgtcttcatcttcccgccatctgatgagcagttgaaatctggaactgcctctgttgtgtgcctgctgaataacttctatcccagagaggccaaagtacagtggaaggtggataacgccctccaatcgggtaactcccaggagagtgtcacagagcaggacagcaaggacagcacctacagcctcagcagcaccctgacgctgagcaaagcagactacgagaaacacaaagtctacgcctgcgaagtcacccatcagggcctgagctcgcccgtcacaaagagcttcaacaggggagagtgt

SEQ ID NO: 12 - protein, 5 aa, Artificial Sequence
  Anti-OX40L antibody VH CDR1
YAWMS

SEQ ID NO: 13 - protein, 5 aa, Artificial Sequence
  Anti-OX40L antibody VH CDR1
DYWMH

SEQ ID NO: 14 - protein, 5 aa, Artificial Sequence
  Anti-OX40L antibody VH CDR1
NYWMQ

SEQ ID NO: 15 - protein, 19 aa, Artificial Sequence
  Anti-OX40L antibody VH CDR2
RIKGEPDGGTTEYADSVKG

SEQ ID NO: 16 - protein, 17 aa, Artificial Sequence
  Anti-OX40L antibody VH CDR2
EIDPPNGRTNYNEKFKS

SEQ ID NO: 17 - protein, 17 aa, Artificial Sequence
  Anti-OX40L antibody VH CDR2
EIDPGNGRTNYNEKFKN

SEQ ID NO: 18 - protein, 17 aa, Artificial Sequence
  Anti-OX40L antibody VH CDR2
EIDPSDGRTNYNEKFKN

SEQ ID NO: 19 - protein, 6 aa, Artificial Sequence
  Anti-OX40L antibody VH CDR3
RRGLDV

SEQ ID NO: 20 - protein, 7 aa, Artificial Sequence
  Anti-OX40L antibody VH CDR3
GIYYVDY

SEQ ID NO: 21 - protein, 9 aa, Artificial Sequence
  Anti-OX40L antibody VH CDR3
EGAGRGFPY

SEQ ID NO: 22 - protein, 9 aa, Artificial Sequence
  Anti-OX40L antibody VH CDR3
EVSLRSMDY

SEQ ID NO: 23 - protein, 11 aa, Artificial Sequence
  Anti-OX40L antibody VL CDR1
RASQSIGRWLA

SEQ ID NO: 24 - protein, 16 aa, Artificial Sequence
  Anti-OX40L antibody VL CDR1
RSSQSLVHSNGNTYLH

SEQ ID NO: 25 - protein, 7 aa, Artificial Sequence
  Anti-OX40L antibody VL CDR2
KATILES

SEQ ID NO: 26 - protein, 7 aa, Artificial Sequence
  Anti-OX40L antibody VL CDR2
KVSNRFS

SEQ ID NO: 27 - protein, 9 aa, Artificial Sequence
  Anti-OX40L antibody VL CDR3
QQYNSYPYT

SEQ ID NO: 28 - protein, 9 aa, Artificial Sequence
  Anti-OX40L antibody VL CDR3
SQSTHVPPT

SEQ ID NO: 29 - protein, 9 aa, Artificial Sequence
  Anti-OX40L antibody VL CDR3
SQSTHVPWT

SEQ ID NO: 30 - protein, 9 aa, Artificial Sequence
  Anti-OX40L antibody VL CDR3
SQSTHVPFT

SEQ ID NO: 31 - protein, 15 aa, Artificial Sequence
  linker 1
GGGGSGGGGSGGGGS

SEQ ID NO: 32 - protein, 20 aa, Artificial Sequence
  linker 2
GGGGSGGGGSGGGGSGGGGS

SEQ ID NO: 33 - protein, 120 aa, Artificial Sequence
  Oxelumab VH
EVQLLESGGGLVQPGGSLRLSCAASGFTFNSYAMSWVRQAPGKGLEWVSIISGSGGFTYYADSVKGRFTISRDNSRTTLYLQMNSLRAEDTAVYYCAKDRLVAPGTFDYWGQGALVTVSS

SEQ ID NO: 34 - protein, 107 aa, Artificial Sequence
  Oxelumab VL
DIQMTQSPSSLSASVGDRVTITCRASQGISSWLAWYQQKPEKAPKSLIYAASSLQSGVPSRFSGSGSGTDFTLTISSLQPEDFATYYCQQYNSYPYTFGQGTKLEIK

SEQ ID NO: 35 - protein, 121 aa, Artificial Sequence [sequence omitted]

SEQ ID NO: 36 - protein, 107 aa, Artificial Sequence [sequence omitted]

SEQ ID NO: 37 - protein, 117 aa, Artificial Sequence
  02C09 VH
QMQLVQSGGGLVKPGGSLRVSCAASGFTFNYAWMSWVRQAPGKGLEWVGRIKGEPDGGTTEYADSVKGRFTISRDNSKNTLYLQMNSLRAEDTAVYYCVSRRGLDVWGQGTTVTVSS

SEQ ID NO: 38 - protein, 107 aa, Artificial Sequence
  02C09 VL
DIQMTQSPSSLSASLGDRVTITCRASQSIGRWLAWYQQKPGNAPKLLIYKATILESGVPSRFSGSGSGTEFALTISSLQPDDFSAYYCQQYNSYPYTFGQGTKLEIK

SEQ ID NO: 39 - DNA, 351 bp, Artificial Sequence
  02C09 VH
caaatgcagcttgttcaatccggcggaggcctggttaagcctggcggatctctgagagtgtcttgtgccgccagcggcttcaccttcaattacgcctggatgagctgggtccgacaggcccctggaaaaggactggaatgggtcggaagaatcaagggcgagcctgatggcggaaccacagagtacgccgatagcgtgaagggcagattcaccatcagccgggacaacagcaagaacaccctgtacctgcagatgaactccctgagagccgaggacacagccgtgtactactgtgtgtctagaagaggcctggatgtgtggggccagggaacaacagtgacagtttcttct

SEQ ID NO: 40 - DNA, 321 bp, Artificial Sequence
  02C09 VL
gatatccagatgacacagagccctagcagcctgtctgcctctctgggcgatagagtgaccatcacatgtcgggccagccagtctattggacggtggctggcctggtatcagcaaaagcctggaaacgcccctaagctgctgatctacaaggccaccatcctggaaagcggagtgccttctagattttctggcagcggctctggcaccgagtttgccctgacaattagctccctgcagcctgacgacttcagcgcctactactgccagcagtacaacagctacccctacaccttcggccagggcacaaagctggaaatcaag

SEQ ID NO: 41 - protein, 116 aa, Artificial Sequence
  hu3F07 VH
QVQLVQSGAEVKKPGASVKVSCKASGFTFPDYWMHWVRQAPGQGLEWMGEIDPPNGRTNYNEKFKSRVTMTRDTSISTAYMELSRLRSDDTAVYYCARGIYYVDYWGQGTTVTVSS

SEQ ID NO: 42 - protein, 112 aa, Artificial Sequence
  hu3F07 VL
DIVMTQSPLSLPVTLGEPASISCRSSQSLVHSNGNTYLHWYLQKPGQSPQLLIYKVSNRFSGVPDRFSGSGSGTDFTLKISRVEAEDVGVYYCSQSTHVPPTFGGGTKLEIK

SEQ ID NO: 43 - DNA, 348 bp, Artificial Sequence
  hu3F07 VH
caagttcaactggttcagtctggcgccgaagtgaagaaaccaggcgccagcgtgaaggtgtcctgcaaggcctctggcttcacattccccgactactggatgcactgggttcgacaggctccaggacagggactcgaatggatgggcgagatcgatcctcctaacggccggaccaactacaacgagaagttcaagagcagagtgaccatgaccagagacaccagcatcagcaccgcctacatggaactgagcagactgagaagcgacgacaccgccgtgtactactgtgccagaggcatctactacgtggactactggggccagggcaccacagtgacagttagctct

SEQ ID NO: 44 - DNA, 336 bp, Artificial Sequence
  hu3F07 VL
gatatcgtgatgacacagagccctctgagcctgcctgtgacactgggagaacctgccagcatcagctgtagaagcagccagagcctggtgcacagcaacggcaatacctacctgcactggtatctgcagaagcccggacagtctccccagctgctgatctacaaggtgtccaacagattcagcggcgtgcccgatagattttctggcagcggctctggcaccgacttcaccctgaagattagcagagtggaagccgaggacgtgggcgtgtactactgtagccagtctacccacgtgccacctacctttggcggcggaacaaagctggaaatcaag

SEQ ID NO: 45 - protein, 118 aa, Artificial Sequence
  10H07 VH
QVYLQQSGAELVKPGASVKLSCKASGYTFTDYWMHWVKQRPGQGLEWIGEIDPGNGRTNYNEKFKNKATLSVDKSSNTAYMQFSSLTSEDSAVFYCASEGAGRGFPYWGQGTLVTVSA

SEQ ID NO: 46 - protein, 112 aa, Artificial Sequence
  10H07 VL
DVVLTQTPLSLPVSLGDQASISCRSSQSLVHSNGNTYLHWYLQKPGQSPKLLIYKVSNRFSGVPDRFSGSGSGTDFTLKISRVEAEDLGVYFCSQSTHVPWTFGGGTKLEIK

SEQ ID NO: 47 - DNA, 354 bp, Artificial Sequence
  10H07 VH
caggtttatctacagcagtctggggctgaactggtgaagcctggggcttcagtgaagctgtcctgcaaggcttctggctacaccttcaccgactactggatgcactgggtgaagcagaggcctggacaaggccttgagtggattggagagattgatcctggcaacggtcgtactaactacaatgagaagttcaagaacaaggccacactgagtgtagacaaatcctccaatacagcctacatgcaattcagcagcctgacatctgaggactctgcggtcttttactgtgcaagcgagggagctggacgtggatttccttactggggccaagggactctggtcactgtctccgca

SEQ ID NO: 48 - DNA, 336 bp, Artificial Sequence
  10H07 VL
gatgttgtgctgacccaaactccactctccctgcctgtcagtcttggagatcaagcctccatctcttgcagatctagtcagagccttgtacacagtaatggaaacacctatttacattggtacctgcagaagccaggccagtctccaaagctcctgatctacaaagtttccaaccgattttctggggtcccagacaggttcagtggcagtggatcagggacagatttcacactcaagatcagcagagtggaggctgaggatctgggagtttatttctgctctcaaagtacacatgttccgtggacgttcggtggaggcaccaagctggaaatcaaa

SEQ ID NO: 49 - protein, 118 aa, Artificial Sequence
  21G07 VH
QVQLQQSGAELVKPGASVKLSCKASGYTFTNYWMQWVKQRPGQGLEWIGEIDPSDGRTNYNEKFKNKATLTVDRSSSTAYIKLSSLTSEDSAVYYCAREVSLRSMDYWGQGTSVTVSS

SEQ ID NO: 50 - protein, 112 aa, Artificial Sequence
  21G07 VL
DIVLTQSPLSLPVSLGDQASISCRSSQSLVHSNGNTYLHWYLQKPGQSPKLLIYKVSNRFSGVPDRFSGSGSGTDFTLKISRVEAEDLGVYFCSQSTHVPFTFGSGTKLEIK

SEQ ID NO: 51 - DNA, 354 bp, Artificial Sequence
  21G07 VH
caggtccaactgcagcagtctggggctgaactggtgaagcctggggcttcagtgaagctgtcctgcaaggcttctggctacaccttcaccaactactggatgcaatgggtgaaacagaggcccggacaaggccttgagtggattggagagattgatcctagcgacggtcgtactaactacaatgagaagttcaagaacaaggccacactgactgtagacagatcctccagcacagcctacataaaactcagcagcctgacatctgaggactctgcggtctattactgtgcaagagaggtttcactacggtcaatggactactggggccaagggacctcagtcaccgtctcctca

SEQ ID NO: 52 - DNA, 336 bp, Artificial Sequence
  21G07 VL
gacattgttctcacccagtctccactctccctgcctgtcagtcttggagatcaagcctccatctcttgcagatctagtcagagccttgtacacagtaatggaaacacctatttacattggtacctgcagaagccaggccagtctccaaagctcctgatctacaaagtttccaaccgattttctggggtcccagacaggttcagtggcagtggatcagggacagatttcacactcaagatcagcagagtggaggctgaggatctgggagtttatttctgctctcaaagtacacatgttccattcacgttcggctcggggacaaagttggaaataaaa

SEQ ID NO: 53 - protein, 116 aa, Artificial Sequence
  I3F07 VH
QIQLAQSGAELVKPGASVKLSCKASGFTFPDYWMHWVKQRPGQGLEWIGEIDPPNGRTNYNEKFKSKATLTVDSSSNTAYMQLSRLTSEDSAVYYCARGIYYVDYWGQGTTLTVSS

SEQ ID NO: 54 - protein, 112 aa, Artificial Sequence
  I3F07 VL
DIVLTQSPLSLPVSLGDQASISCRSSQSLVHSNGNTYLHWYLQKPGQSPKLLIYKVSNRFSGVPDRFSGSGSGTDFTLKISRVEAEDLGVYFCSQSTHVPPTFGGGSKLEIK

SEQ ID NO: 55 - DNA, 348 bp, Artificial Sequence
  I3F07 VH
cagattcagctggctcagtctggcgccgaacttgtgaaacctggcgcctctgtgaagctgagctgcaaggccagcggcttcacctttcctgactactggatgcactgggtcaagcagaggcctggacagggactcgaatggatcggcgagatcgatcctcctaacggccggaccaactacaacgagaagttcaagagcaaggccacactgaccgtggacagcagcagcaataccgcctacatgcagctgagcagactgacctctgaggacagcgccgtgtactactgtgccagaggcatctactacgtggactactggggccagggcacaaccctgacagtttcttct

SEQ ID NO: 56 - DNA, 336 bp, Artificial Sequence
  I3F07 VL
gatatcgtgctgacacagagccctctgagcctgcctgtttctctgggagatcaggccagcatcagctgcagatcctctcagagcctggtgcacagcaacggcaatacctacctgcactggtatctgcagaagcccggccagtctcctaagctgctgatctacaaggtgtccaacaggttcagcggcgtgcccgatagattttctggctctggcagcggcaccgacttcaccctgaagatttctagagtggaagccgaggacctgggcgtgtacttctgttctcagtctacccacgtgccacctacctttggcggcggaagcaagctggaaatcaag

SEQ ID NO: 57 - protein, 707 aa, Artificial Sequence
  02C09-TNFai HC heavy chain
QMQLVQSGGGLVKPGGSLRVSCAASGFTFNYAWMSWVRQAPGKGLEWVGRIKGEPDGGTTEYADSVKGRFTISRDNSKNTLYLQMNSLRAEDTAVYYCVSRRGLDVWGQGTTVTVSSASTKGPSVFPLAPCSRSTSESTAALGCLVKDYFPEPVTVSWNSGALTSGVHTFPAVLQSSGLYSLSSVVTVPSSSLGTKTYTCNVDHKPSNTKVDKRVESKYGPPCPPCPAPEFLGGPSVFLFPPKPKDTLMISRTPEVTCVVVDVSQEDPEVQFNWYVDGVEVHNAKTKPREEQFNSTYRVVSVLTVLHQDWLNGKEYKCKVSNKGLPSSIEKTISKAKGQPREPQVYTLPPSQEEMTKNQVSLTCLVKGFYPSDIAVEWESNGQPENNYKTTPPVLDSDGSFFLYSRLTVDKSRWQEGNVFSCSVMHEALHNHYTQKSLSLSLGKGGGGSGGGGSGGGGSEVQLVESGGGLVQPGRSLRLSCAASGFTFDDYAMHWVRQAPGKGLEWVSAITWNSGHIDYADSVEGRFTISRDNAKNSLYLQMNSLRAEDTAVYYCAKVSYLSTASSLDYWGQGTLVTVSSGGGGSGGGGSGGGGSGGGGSDIQMTQSPSSLSASVGDRVTITCRASQGIRNYLAWYQQKPGKAPKLLIYAASTLQSGVPSRFSGSGSGTDFTLTISSLQPEDVATYYCQRYNRAPYTFGQGTKVEIK

SEQ ID NO: 58 - DNA, 2121 bp, Artificial Sequence
  02C09-TNFai HC heavy chain
caaatgcagcttgttcaatccggcggaggcctggttaagcctggcggatctctgagagtgtcttgtgccgccagcggcttcaccttcaattacgcctggatgagctgggtccgacaggcccctggaaaaggactggaatgggtcggaagaatcaagggcgagcctgatggcggaaccacagagtacgccgatagcgtgaagggcagattcaccatcagccgggacaacagcaagaacaccctgtacctgcagatgaactccctgagagccgaggacacagccgtgtactactgtgtgtctagaagaggcctggatgtgtggggccagggaacaacagtgacagtttcttctgcttccaccaagggcccatccgtcttccccctggcgccctgctccaggagcacctccgagagcacagccgccctgggctgcctggtcaaggactacttccccgaaccggtgacggtgtcgtggaactcaggcgccctgaccagcggcgtgcacaccttcccggctgtcctacagtcctcaggactctactccctcagcagcgtggtgaccgtgccctccagcagcttgggcacgaagacctacacctgcaacgtagatcacaagcccagcaacaccaaggtggacaagagagttgagtccaaatatggtcccccatgcccaccatgcccagcacctgagttcctggggggaccatcagtcttcctgttccccccaaaacccaaggacactctcatgatctcccggacccctgaggtcacgtgcgtggtggtggacgtgagccaggaagaccccgaggtccagttcaactggtacgtggatggcgtggaggtgcataatgccaagacaaagccgcgggaggagcagttcaacagcacgtaccgtgtggtcagcgtcctcaccgtcctgcaccaggactggctgaacggcaaggagtacaagtgcaaggtctccaacaaaggcctcccgtcctccatcgagaaaaccatctccaaagccaaagggcagccccgagagccacaggtgtacaccctgcccccatcccaggaggagatgaccaagaaccaggtcagcctgacctgcctggtcaaaggcttctaccccagcgacatcgccgtggagtgggagagcaatgggcagccggagaacaactacaagaccacgcctcccgtgctggactccgacggctccttcttcctctacagcaggctaaccgtggacaagagcaggtggcaggaggggaatgtcttctcatgctccgtgatgcatgaggctctgcacaaccactacacacagaagagcctctccctgtctctgggtaaaggtggtggcggatctggcggcggaggaagcggaggcggaggctccgaagtgcaactggttgaatctggcggaggactggtgcagcctggaagaagcctgagactgtcttgtgccgccagcggcttcaccttcgatgattatgccatgcactgggtccgacaggcccctggaaaaggacttgaatgggtgtccgccatcacctggaacagcggccacatcgattacgccgatagcgtggaaggccggttcaccatcagcagagacaacgccaagaacagcctgtacctgcagatgaactccctgagagccgaggacaccgccgtgtactactgtgccaaagtgtcttacctgagcaccgcctccagcctggattattggggacagggcacactggtcacagtgtcctctggtggcggaggttctggcggaggtggtagtggtggcggtggaagtggtggcggcggatctgatatccagatgacacagagccctagcagcctgtctgcctctgtgggcgatagagtgaccatcacctgtagagccagccagggcatcagaaactacctggcctggtatcagcagaagcccggaaaggcccctaagctgctgatctatgccgcctctacactgcagagcggcgtgccatctagattttctggcagcggctctggcaccgacttcaccctgacaatttctagcctgcagcctgaggacgtggccacctactactgccagagatacaacagagccccttacaccttcggccagggcaccaaggtggaaatcaag

SEQ ID NO: 59 - protein, 477 aa, Artificial Sequence
  02C09-TNFai LC light chain
DIQMTQSPSSLSASLGDRVTITCRASQSIGRWLAWYQQKPGNAPKLLIYKATILESGVPSRFSGSGSGTEFALTISSLQPDDFSAYYCQQYNSYPYTFGQGTKLEIKRTVAAPSVFIFPPSDEQLKSGTASVVCLLNNFYPREAKVQWKVDNALQSGNSQESVTEQDSKDSTYSLSSTLTLSKADYEKHKVYACEVTHQGLSSPVTKSFNRGECGGGGSGGGGSGGGGSEVQLVESGGGLVQPGRSLRLSCAASGFTFDDYAMHWVRQAPGKGLEWVSAITWNSGHIDYADSVEGRFTISRDNAKNSLYLQMNSLRAEDTAVYYCAKVSYLSTASSLDYWGQGTLVTVSSGGGGSGGGGSGGGGSGGGGSDIQMTQSPSSLSASVGDRVTITCRASQGIRNYLAWYQQKPGKAPKLLIYAASTLQSGVPSRFSGSGSGTDFTLTISSLQPEDVATYYCQRYNRAPYTFGQGTKVEIK

SEQ ID NO: 60 - DNA, 1431 bp, Artificial Sequence
  02C09-TNFai LC light chain
gatatccagatgacacagagccctagcagcctgtctgcctctctgggcgatagagtgaccatcacatgtcgggccagccagtctattggacggtggctggcctggtatcagcaaaagcctggaaacgcccctaagctgctgatctacaaggccaccatcctggaaagcggagtgccttctagattttctggcagcggctctggcaccgagtttgccctgacaattagctccctgcagcctgacgacttcagcgcctactactgccagcagtacaacagctacccctacaccttcggccagggcacaaagctggaaatcaagcgtacggtggcggcgccatctgtcttcatcttcccgccatctgatgagcagttgaaatctggaactgcctctgttgtgtgcctgctgaataacttctatcccagagaggccaaagtacagtggaaggtggataacgccctccaatcgggtaactcccaggagagtgtcacagagcaggacagcaaggacagcacctacagcctcagcagcaccctgacgctgagcaaagcagactacgagaaacacaaagtctacgcctgcgaagtcacccatcagggcctgagctcgcccgtcacaaagagcttcaacaggggagagtgtggtggtggcggatctggcggcggaggaagcggaggcggaggctccgaagtgcaactggttgaatctggcggaggactggtgcagcctggaagaagcctgagactgtcttgtgccgccagcggcttcaccttcgatgattatgccatgcactgggtccgacaggcccctggaaaaggacttgaatgggtgtccgccatcacctggaacagcggccacatcgattacgccgatagcgtggaaggccggttcaccatcagcagagacaacgccaagaacagcctgtacctgcagatgaactccctgagagccgaggacaccgccgtgtactactgtgccaaagtgtcttacctgagcaccgcctccagcctggattattggggacagggcacactggtcacagtgtcctctggtggcggaggttctggcggaggtggtagtggtggcggtggaagtggtggcggcggatctgatatccagatgacacagagccctagcagcctgtctgcctctgtgggcgatagagtgaccatcacctgtagagccagccagggcatcagaaactacctggcctggtatcagcagaagcccggaaaggcccctaagctgctgatctatgccgcctctacactgcagagcggcgtgccatctagattttctggcagcggctctggcaccgacttcaccctgacaatttctagcctgcagcctgaggacgtggccacctactactgccagagatacaacagagccccttacaccttcggccagggcaccaaggtggaaatcaag

SEQ ID NO: 61 - protein, 706 aa, Artificial Sequence
  Hu3F07-TNFai HC heavy chain
QVQLVQSGAEVKKPGASVKVSCKASGFTFPDYWMHWVRQAPGQGLEWMGEIDPPNGRTNYNEKFKSRVTMTRDTSISTAYMELSRLRSDDTAVYYCARGIYYVDYWGQGTTVTVSSASTKGPSVFPLAPCSRSTSESTAALGCLVKDYFPEPVTVSWNSGALTSGVHTFPAVLQSSGLYSLSSVVTVPSSSLGTKTYTCNVDHKPSNTKVDKRVESKYGPPCPPCPAPEFLGGPSVFLFPPKPKDTLMISRTPEVTCVVVDVSQEDPEVQFNWYVDGVEVHNAKTKPREEQFNSTYRVVSVLTVLHQDWLNGKEYKCKVSNKGLPSSIEKTISKAKGQPREPQVYTLPPSQEEMTKNQVSLTCLVKGFYPSDIAVEWESNGQPENNYKTTPPVLDSDGSFFLYSRLTVDKSRWQEGNVFSCSVMHEALHNHYTQKSLSLSLGKGGGGSGGGGSGGGGSEVQLVESGGGLVQPGRSLRLSCAASGFTFDDYAMHWVRQAPGKGLEWVSAITWNSGHIDYADSVEGRFTISRDNAKNSLYLQMNSLRAEDTAVYYCAKVSYLSTASSLDYWGQGTLVTVSSGGGGSGGGGSGGGGSGGGGSDIQMTQSPSSLSASVGDRVTITCRASQGIRNYLAWYQQKPGKAPKLLIYAASTLQSGVPSRFSGSGSGTDFTLTISSLQPEDVATYYCQRYNRAPYTFGQGTKVEIK

SEQ ID NO: 62 - DNA, 2118 bp, Artificial Sequence
  Hu3F07-TNFai HC heavy chain
caagttcaactggttcagtctggcgccgaagtgaagaaaccaggcgccagcgtgaaggtgtcctgcaaggcctctggcttcacattccccgactactggatgcactgggttcgacaggctccaggacagggactcgaatggatgggcgagatcgatcctcctaacggccggaccaactacaacgagaagttcaagagcagagtgaccatgaccagagacaccagcatcagcaccgcctacatggaactgagcagactgagaagcgacgacaccgccgtgtactactgtgccagaggcatctactacgtggactactggggccagggcaccacagtgacagttagctctgcttccaccaagggcccatccgtcttccccctggcgccctgctccaggagcacctccgagagcacagccgccctgggctgcctggtcaaggactacttccccgaaccggtgacggtgtcgtggaactcaggcgccctgaccagcggcgtgcacaccttcccggctgtcctacagtcctcaggactctactccctcagcagcgtggtgaccgtgccctccagcagcttgggcacgaagacctacacctgcaacgtagatcacaagcccagcaacaccaaggtggacaagagagttgagtccaaatatggtcccccatgcccaccatgcccagcacctgagttcctggggggaccatcagtcttcctgttccccccaaaacccaaggacactctcatgatctcccggacccctgaggtcacgtgcgtggtggtggacgtgagccaggaagaccccgaggtccagttcaactggtacgtggatggcgtggaggtgcataatgccaagacaaagccgcgggaggagcagttcaacagcacgtaccgtgtggtcagcgtcctcaccgtcctgcaccaggactggctgaacggcaaggagtacaagtgcaaggtctccaacaaaggcctcccgtcctccatcgagaaaaccatctccaaagccaaagggcagccccgagagccacaggtgtacaccctgcccccatcccaggaggagatgaccaagaaccaggtcagcctgacctgcctggtcaaaggcttctaccccagcgacatcgccgtggagtgggagagcaatgggcagccggagaacaactacaagaccacgcctcccgtgctggactccgacggctccttcttcctctacagcaggctaaccgtggacaagagcaggtggcaggaggggaatgtcttctcatgctccgtgatgcatgaggctctgcacaaccactacacacagaagagcctctccctgtctctgggtaaaggtggtggcggatctggcggcggaggaagcggaggcggaggctccgaagtgcaactggttgaatctggcggaggactggtgcagcctggaagaagcctgagactgtcttgtgccgccagcggcttcaccttcgatgattatgccatgcactgggtccgacaggcccctggaaaaggacttgaatgggtgtccgccatcacctggaacagcggccacatcgattacgccgatagcgtggaaggccggttcaccatcagcagagacaacgccaagaacagcctgtacctgcagatgaactccctgagagccgaggacaccgccgtgtactactgtgccaaagtgtcttacctgagcaccgcctccagcctggattattggggacagggcacactggtcacagtgtcctctggtggcggaggttctggcggaggtggtagtggtggcggtggaagtggtggcggcggatctgatatccagatgacacagagccctagcagcctgtctgcctctgtgggcgatagagtgaccatcacctgtagagccagccagggcatcagaaactacctggcctggtatcagcagaagcccggaaaggcccctaagctgctgatctatgccgcctctacactgcagagcggcgtgccatctagattttctggcagcggctctggcaccgacttcaccctgacaatttctagcctgcagcctgaggacgtggccacctactactgccagagatacaacagagccccttacaccttcggccagggcaccaaggtggaaatcaag

SEQ ID NO: 63 - protein, 482 aa, Artificial Sequence
  Hu3F07-TNFai LC light chain
DIVMTQSPLSLPVTLGEPASISCRSSQSLVHSNGNTYLHWYLQKPGQSPQLLIYKVSNRFSGVPDRFSGSGSGTDFTLKISRVEAEDVGVYYCSQSTHVPPTFGGGTKLEIKRTVAAPSVFIFPPSDEQLKSGTASVVCLLNNFYPREAKVQWKVDNALQSGNSQESVTEQDSKDSTYSLSSTLTLSKADYEKHKVYACEVTHQGLSSPVTKSFNRGECGGGGSGGGGSGGGGSEVQLVESGGGLVQPGRSLRLSCAASGFTFDDYAMHWVRQAPGKGLEWVSAITWNSGHIDYADSVEGRFTISRDNAKNSLYLQMNSLRAEDTAVYYCAKVSYLSTASSLDYWGQGTLVTVSSGGGGSGGGGSGGGGSGGGGSDIQMTQSPSSLSASVGDRVTITCRASQGIRNYLAWYQQKPGKAPKLLIYAASTLQSGVPSRFSGSGSGTDFTLTISSLQPEDVATYYCQRYNRAPYTFGQGTKVEIK

SEQ ID NO: 64 - DNA, 1446 bp, Artificial Sequence
  Hu3F07-TNFai LC light chain
gatatcgtgatgacacagagccctctgagcctgcctgtgacactgggagaacctgccagcatcagctgtagaagcagccagagcctggtgcacagcaacggcaatacctacctgcactggtatctgcagaagcccggacagtctccccagctgctgatctacaaggtgtccaacagattcagcggcgtgcccgatagattttctggcagcggctctggcaccgacttcaccctgaagattagcagagtggaagccgaggacgtgggcgtgtactactgtagccagtctacccacgtgccacctacctttggcggcggaacaaagctggaaatcaagcgtacggtggcggcgccatctgtcttcatcttcccgccatctgatgagcagttgaaatctggaactgcctctgttgtgtgcctgctgaataacttctatcccagagaggccaaagtacagtggaaggtggataacgccctccaatcgggtaactcccaggagagtgtcacagagcaggacagcaaggacagcacctacagcctcagcagcaccctgacgctgagcaaagcagactacgagaaacacaaagtctacgcctgcgaagtcacccatcagggcctgagctcgcccgtcacaaagagcttcaacaggggagagtgtggtggtggcggatctggcggcggaggaagcggaggcggaggctccgaagtgcaactggttgaatctggcggaggactggtgcagcctggaagaagcctgagactgtcttgtgccgccagcggcttcaccttcgatgattatgccatgcactgggtccgacaggcccctggaaaaggacttgaatgggtgtccgccatcacctggaacagcggccacatcgattacgccgatagcgtggaaggccggttcaccatcagcagagacaacgccaagaacagcctgtacctgcagatgaactccctgagagccgaggacaccgccgtgtactactgtgccaaagtgtcttacctgagcaccgcctccagcctggattattggggacagggcacactggtcacagtgtcctctggtggcggaggttctggcggaggtggtagtggtggcggtggaagtggtggcggcggatctgatatccagatgacacagagccctagcagcctgtctgcctctgtgggcgatagagtgaccatcacctgtagagccagccagggcatcagaaactacctggcctggtatcagcagaagcccggaaaggcccctaagctgctgatctatgccgcctctacactgcagagcggcgtgccatctagattttctggcagcggctctggcaccgacttcaccctgacaatttctagcctgcagcctgaggacgtggccacctactactgccagagatacaacagagccccttacaccttcggccagggcaccaaggtggaaatcaag

SEQ ID NO: 65 - protein, 707 aa, Artificial Sequence
  TNFai-02C09 HC heavy chain
EVQLVESGGGLVQPGRSLRLSCAASGFTFDDYAMHWVRQAPGKGLEWVSAITWNSGHIDYADSVEGRFTISRDNAKNSLYLQMNSLRAEDTAVYYCAKVSYLSTASSLDYWGQGTLVTVSSASTKGPSVFPLAPCSRSTSESTAALGCLVKDYFPEPVTVSWNSGALTSGVHTFPAVLQSSGLYSLSSVVTVPSSSLGTKTYTCNVDHKPSNTKVDKRVESKYGPPCPPCPAPEFLGGPSVFLFPPKPKDTLMISRTPEVTCVVVDVSQEDPEVQFNWYVDGVEVHNAKTKPREEQFNSTYRVVSVLTVLHQDWLNGKEYKCKVSNKGLPSSIEKTISKAKGQPREPQVYTLPPSQEEMTKNQVSLTCLVKGFYPSDIAVEWESNGQPENNYKTTPPVLDSDGSFFLYSRLTVDKSRWQEGNVFSCSVMHEALHNHYTQKSLSLSLGKGGGGSGGGGSGGGGSQMQLVQSGGGLVKPGGSLRVSCAASGFTFNYAWMSWVRQAPGKGLEWVGRIKGEPDGGTTEYADSVKGRFTISRDNSKNTLYLQMNSLRAEDTAVYYCVSRRGLDVWGQGTTVTVSSGGGGSGGGGSGGGGSGGGGSDIQMTQSPSSLSASLGDRVTITCRASQSIGRWLAWYQQKPGNAPKLLIYKATILESGVPSRFSGSGSGTEFALTISSLQPDDFSAYYCQQYNSYPYTFGQGTKLEIK

SEQ ID NO: 66 - DNA, 2121 bp, Artificial Sequence
  TNFai-02C09 HC heavy chain
gaagtgcaactggttgaatctggcggaggactggtgcagcctggaagaagcctgagactgtcttgtgccgccagcggcttcaccttcgatgattatgccatgcactgggtccgacaggcccctggaaaaggacttgaatgggtgtccgccatcacctggaacagcggccacatcgattacgccgatagcgtggaaggccggttcaccatcagcagagacaacgccaagaacagcctgtacctgcagatgaactccctgagagccgaggacaccgccgtgtactactgtgccaaagtgtcttacctgagcaccgcctccagcctggattattggggacagggcacactggtcacagtgtcctctgcttccaccaagggcccatccgtcttccccctggcgccctgctccaggagcacctccgagagcacagccgccctgggctgcctggtcaaggactacttccccgaaccggtgacggtgtcgtggaactcaggcgccctgaccagcggcgtgcacaccttcccggctgtcctacagtcctcaggactctactccctcagcagcgtggtgaccgtgccctccagcagcttgggcacgaagacctacacctgcaacgtagatcacaagcccagcaacaccaaggtggacaagagagttgagtccaaatatggtcccccatgcccaccatgcccagcacctgagttcctggggggaccatcagtcttcctgttccccccaaaacccaaggacactctcatgatctcccggacccctgaggtcacgtgcgtggtggtggacgtgagccaggaagaccccgaggtccagttcaactggtacgtggatggcgtggaggtgcataatgccaagacaaagccgcgggaggagcagttcaacagcacgtaccgtgtggtcagcgtcctcaccgtcctgcaccaggactggctgaacggcaaggagtacaagtgcaaggtctccaacaaaggcctcccgtcctccatcgagaaaaccatctccaaagccaaagggcagccccgagagccacaggtgtacaccctgcccccatcccaggaggagatgaccaagaaccaggtcagcctgacctgcctggtcaaaggcttctaccccagcgacatcgccgtggagtgggagagcaatgggcagccggagaacaactacaagaccacgcctcccgtgctggactccgacggctccttcttcctctacagcaggctaaccgtggacaagagcaggtggcaggaggggaatgtcttctcatgctccgtgatgcatgaggctctgcacaaccactacacacagaagagcctctccctgtctctgggtaaaggtggtggcggatctggcggcggaggaagcggaggcggaggatcccaaatgcagcttgttcaatccggcggaggcctggttaagcctggcggatctctgagagtgtcttgtgccgccagcggcttcaccttcaattacgcctggatgagctgggtccgacaggcccctggaaaaggactggaatgggtcggaagaatcaagggcgagcctgatggcggaaccacagagtacgccgatagcgtgaagggcagattcaccatcagccgggacaacagcaagaacaccctgtacctgcagatgaactccctgagagccgaggacacagccgtgtactactgtgtgtctagaagaggcctggatgtgtggggccagggaacaacagtgacagtttcttctggtggcggaggttctggcggaggtggtagtggtggcggtggaagtggtggcggcggatctgatatccagatgacacagagccctagcagcctgtctgcctctctgggcgatagagtgaccatcacatgtcgggccagccagtctattggacggtggctggcctggtatcagcaaaagcctggaaacgcccctaagctgctgatctacaaggccaccatcctggaaagcggagtgccttctagattttctggcagcggctctggcaccgagtttgccctgacaattagctccctgcagcctgacgacttcagcgcctactactgccagcagtacaacagctacccctacaccttcggccagggcacaaagctggaaatcaag

SEQ ID NO: 67 - protein, 473 aa, Artificial Sequence
  TNFai-02C09 LC light chain
DIQMTQSPSSLSASVGDRVTITCRASQGIRNYLAWYQQKPGKAPKLLIYAASTLQSGVPSRFSGSGSGTDFTLTISSLQPEDVATYYCQRYNRAPYTFGQGTKVEIKRTVAAPSVFIFPPSDEQLKSGTASVVCLLNNFYPREAKVQWKVDNALQSGNSQESVTEQDSKDSTYSLSSTLTLSKADYEKHKVYACEVTHQGLSSPVTKSFNRGECGGGGSGGGGSGGGGSQMQLVQSGGGLVKPGGSLRVSCAASGFTFNYAWMSWVRQAPGKGLEWVGRIKGEPDGGTTEYADSVKGRFTISRDNSKNTLYLQMNSLRAEDTAVYYCVSRRGLDVWGQGTTVTVSSGGGGSGGGGSGGGGSGGGGSDIQMTQSPSSLSASLGDRVTITCRASQSIGRWLAWYQQKPGNAPKLLIYKATILESGVPSRFSGSGSGTEFALTISSLQPDDFSAYYCQQYNSYPYTFGQGTKLEIK

SEQ ID NO: 68 - DNA, 1419 bp, Artificial Sequence
  TNFai-02C09 LC light chain
gatatccagatgacacagagccctagcagcctgtctgcctctgtgggcgatagagtgaccatcacctgtagagccagccagggcatcagaaactacctggcctggtatcagcagaagcccggaaaggcccctaagctgctgatctatgccgcctctacactgcagagcggcgtgccatctagattttctggcagcggctctggcaccgacttcaccctgacaatttctagcctgcagcctgaggacgtggccacctactactgccagagatacaacagagccccttacaccttcggccagggcaccaaggtggaaatcaagcgtacggtggcggcgccatctgtcttcatcttcccgccatctgatgagcagttgaaatctggaactgcctctgttgtgtgcctgctgaataacttctatcccagagaggccaaagtacagtggaaggtggataacgccctccaatcgggtaactcccaggagagtgtcacagagcaggacagcaaggacagcacctacagcctcagcagcaccctgacgctgagcaaagcagactacgagaaacacaaagtctacgcctgcgaagtcacccatcagggcctgagctcgcccgtcacaaagagcttcaacaggggagagtgtggtggtggcggatctggcggcggaggaagcggaggcggaggatcccaaatgcagcttgttcaatccggcggaggcctggttaagcctggcggatctctgagagtgtcttgtgccgccagcggcttcaccttcaattacgcctggatgagctgggtccgacaggcccctggaaaaggactggaatgggtcggaagaatcaagggcgagcctgatggcggaaccacagagtacgccgatagcgtgaagggcagattcaccatcagccgggacaacagcaagaacaccctgtacctgcagatgaactccctgagagccgaggacacagccgtgtactactgtgtgtctagaagaggcctggatgtgtggggccagggaacaacagtgacagtttcttctggtggcggaggttctggcggaggtggtagtggtggcggtggaagtggtggcggcggatctgatatccagatgacacagagccctagcagcctgtctgcctctctgggcgatagagtgaccatcacatgtcgggccagccagtctattggacggtggctggcctggtatcagcaaaagcctggaaacgcccctaagctgctgatctacaaggccaccatcctggaaagcggagtgccttctagattttctggcagcggctctggcaccgagtttgccctgacaattagctccctgcagcctgacgacttcagcgcctactactgccagcagtacaacagctacccctacaccttcggccagggcacaaagctggaaatcaag

SEQ ID NO: 69 - protein, 711 aa, Artificial Sequence
  TNFai-hu3F07 HC heavy chain
EVQLVESGGGLVQPGRSLRLSCAASGFTFDDYAMHWVRQAPGKGLEWVSAITWNSGHIDYADSVEGRFTISRDNAKNSLYLQMNSLRAEDTAVYYCAKVSYLSTASSLDYWGQGTLVTVSSASTKGPSVFPLAPCSRSTSESTAALGCLVKDYFPEPVTVSWNSGALTSGVHTFPAVLQSSGLYSLSSVVTVPSSSLGTKTYTCNVDHKPSNTKVDKRVESKYGPPCPPCPAPEFLGGPSVFLFPPKPKDTLMISRTPEVTCVVVDVSQEDPEVQFNWYVDGVEVHNAKTKPREEQFNSTYRVVSVLTVLHQDWLNGKEYKCKVSNKGLPSSIEKTISKAKGQPREPQVYTLPPSQEEMTKNQVSLTCLVKGFYPSDIAVEWESNGQPENNYKTTPPVLDSDGSFFLYSRLTVDKSRWQEGNVFSCSVMHEALHNHYTQKSLSLSLGKGGGGSGGGGSGGGGSQVQLVQSGAEVKKPGASVKVSCKASGFTFPDYWMHWVRQAPGQGLEWMGEIDPPNGRTNYNEKFKSRVTMTRDTSISTAYMELSRLRSDDTAVYYCARGIYYVDYWGQGTTVTVSSGGGGSGGGGSGGGGSGGGGSDIVMTQSPLSLPVTLGEPASISCRSSQSLVHSNGNTYLHWYLQKPGQSPQLLIYKVSNRFSGVPDRFSGSGSGTDFTLKISRVEAEDVGVYYCSQSTHVPPTFGGGTKLEIK

SEQ ID NO: 70 - DNA, 2133 bp, Artificial Sequence
  TNFai-hu3F07 HC heavy chain
gaagtgcaactggttgaatctggcggaggactggtgcagcctggaagaagcctgagactgtcttgtgccgccagcggcttcaccttcgatgattatgccatgcactgggtccgacaggcccctggaaaaggacttgaatgggtgtccgccatcacctggaacagcggccacatcgattacgccgatagcgtggaaggccggttcaccatcagcagagacaacgccaagaacagcctgtacctgcagatgaactccctgagagccgaggacaccgccgtgtactactgtgccaaagtgtcttacctgagcaccgcctccagcctggattattggggacagggcacactggtcacagtgtcctctgcttccaccaagggcccatccgtcttccccctggcgccctgctccaggagcacctccgagagcacagccgccctgggctgcctggtcaaggactacttccccgaaccggtgacggtgtcgtggaactcaggcgccctgaccagcggcgtgcacaccttcccggctgtcctacagtcctcaggactctactccctcagcagcgtggtgaccgtgccctccagcagcttgggcacgaagacctacacctgcaacgtagatcacaagcccagcaacaccaaggtggacaagagagttgagtccaaatatggtcccccatgcccaccatgcccagcacctgagttcctggggggaccatcagtcttcctgttccccccaaaacccaaggacactctcatgatctcccggacccctgaggtcacgtgcgtggtggtggacgtgagccaggaagaccccgaggtccagttcaactggtacgtggatggcgtggaggtgcataatgccaagacaaagccgcgggaggagcagttcaacagcacgtaccgtgtggtcagcgtcctcaccgtcctgcaccaggactggctgaacggcaaggagtacaagtgcaaggtctccaacaaaggcctcccgtcctccatcgagaaaaccatctccaaagccaaagggcagccccgagagccacaggtgtacaccctgcccccatcccaggaggagatgaccaagaaccaggtcagcctgacctgcctggtcaaaggcttctaccccagcgacatcgccgtggagtgggagagcaatgggcagccggagaacaactacaagaccacgcctcccgtgctggactccgacggctccttcttcctctacagcaggctaaccgtggacaagagcaggtggcaggaggggaatgtcttctcatgctccgtgatgcatgaggctctgcacaaccactacacacagaagagcctctccctgtctctgggtaaaggtggtggcggatctggcggcggaggaagcggaggcggaggatcccaagttcaactggttcagtctggcgccgaagtgaagaaaccaggcgccagcgtgaaggtgtcctgcaaggcctctggcttcacattccccgactactggatgcactgggttcgacaggctccaggacagggactcgaatggatgggcgagatcgatcctcctaacggccggaccaactacaacgagaagttcaagagcagagtgaccatgaccagagacaccagcatcagcaccgcctacatggaactgagcagactgagaagcgacgacaccgccgtgtactactgtgccagaggcatctactacgtggactactggggccagggcaccacagtgacagttagctctggtggcggaggttctggcggaggtggtagtggtggcggtggaagtggtggcggcggatctgatatcgtgatgacacagagccctctgagcctgcctgtgacactgggagaacctgccagcatcagctgtagaagcagccagagcctggtgcacagcaacggcaatacctacctgcactggtatctgcagaagcccggacagtctccccagctgctgatctacaaggtgtccaacagattcagcggcgtgcccgatagattttctggcagcggctctggcaccgacttcaccctgaagattagcagagtggaagccgaggacgtgggcgtgtactactgtagccagtctacccacgtgccacctacctttggcggcggaacaaagctggaaatcaag

SEQ ID NO: 71 - protein, 477 aa, Artificial Sequence
  TNFai- hu3F07 LC light chain
DIQMTQSPSSLSASVGDRVTITCRASQGIRNYLAWYQQKPGKAPKLLIYAASTLQSGVPSRFSGSGSGTDFTLTISSLQPEDVATYYCQRYNRAPYTFGQGTKVEIKRTVAAPSVFIFPPSDEQLKSGTASVVCLLNNFYPREAKVQWKVDNALQSGNSQESVTEQDSKDSTYSLSSTLTLSKADYEKHKVYACEVTHQGLSSPVTKSFNRGECGGGGSGGGGSGGGGSQVQLVQSGAEVKKPGASVKVSCKASGFTFPDYWMHWVRQAPGQGLEWMGEIDPPNGRTNYNEKFKSRVTMTRDTSISTAYMELSRLRSDDTAVYYCARGIYYVDYWGQGTTVTVSSGGGGSGGGGSGGGGSGGGGSDIVMTQSPLSLPVTLGEPASISCRSSQSLVHSNGNTYLHWYLQKPGQSPQLLIYKVSNRFSGVPDRFSGSGSGTDFTLKISRVEAEDVGVYYCSQSTHVPPTFGGGTKLEIK

SEQ ID NO: 72 - DNA, 1431 bp, Artificial Sequence
  TNFai- hu3F07 LC light chain
gatatccagatgacacagagccctagcagcctgtctgcctctgtgggcgatagagtgaccatcacctgtagagccagccagggcatcagaaactacctggcctggtatcagcagaagcccggaaaggcccctaagctgctgatctatgccgcctctacactgcagagcggcgtgccatctagattttctggcagcggctctggcaccgacttcaccctgacaatttctagcctgcagcctgaggacgtggccacctactactgccagagatacaacagagccccttacaccttcggccagggcaccaaggtggaaatcaagcgtacggtggcggcgccatctgtcttcatcttcccgccatctgatgagcagttgaaatctggaactgcctctgttgtgtgcctgctgaataacttctatcccagagaggccaaagtacagtggaaggtggataacgccctccaatcgggtaactcccaggagagtgtcacagagcaggacagcaaggacagcacctacagcctcagcagcaccctgacgctgagcaaagcagactacgagaaacacaaagtctacgcctgcgaagtcacccatcagggcctgagctcgcccgtcacaaagagcttcaacaggggagagtgtggtggtggcggatctggcggcggaggaagcggaggcggaggatcccaagttcaactggttcagtctggcgccgaagtgaagaaaccaggcgccagcgtgaaggtgtcctgcaaggcctctggcttcacattccccgactactggatgcactgggttcgacaggctccaggacagggactcgaatggatgggcgagatcgatcctcctaacggccggaccaactacaacgagaagttcaagagcagagtgaccatgaccagagacaccagcatcagcaccgcctacatggaactgagcagactgagaagcgacgacaccgccgtgtactactgtgccagaggcatctactacgtggactactggggccagggcaccacagtgacagttagctctggtggcggaggttctggcggaggtggtagtggtggcggtggaagtggtggcggcggatctgatatcgtgatgacacagagccctctgagcctgcctgtgacactgggagaacctgccagcatcagctgtagaagcagccagagcctggtgcacagcaacggcaatacctacctgcactggtatctgcagaagcccggacagtctccccagctgctgatctacaaggtgtccaacagattcagcggcgtgcccgatagattttctggcagcggctctggcaccgacttcaccctgaagattagcagagtggaagccgaggacgtgggcgtgtactactgtagccagtctacccacgtgccacctacctttggcggcggaacaaagctggaaatcaag

SEQ ID NO: 73 - protein, 706 aa, Artificial Sequence
  I3F07-TNFai HC heavy chain
QIQLAQSGAELVKPGASVKLSCKASGFTFPDYWMHWVKQRPGQGLEWIGEIDPPNGRTNYNEKFKSKATLTVDSSSNTAYMQLSRLTSEDSAVYYCARGIYYVDYWGQGTTLTVSSASTKGPSVFPLAPCSRSTSESTAALGCLVKDYFPEPVTVSWNSGALTSGVHTFPAVLQSSGLYSLSSVVTVPSSSLGTKTYTCNVDHKPSNTKVDKRVESKYGPPCPPCPAPEFLGGPSVFLFPPKPKDTLMISRTPEVTCVVVDVSQEDPEVQFNWYVDGVEVHNAKTKPREEQFNSTYRVVSVLTVLHQDWLNGKEYKCKVSNKGLPSSIEKTISKAKGQPREPQVYTLPPSQEEMTKNQVSLTCLVKGFYPSDIAVEWESNGQPENNYKTTPPVLDSDGSFFLYSRLTVDKSRWQEGNVFSCSVMHEALHNHYTQKSLSLSLGKGGGGSGGGGSGGGGSEVQLVESGGGLVQPGRSLRLSCAASGFTFDDYAMHWVRQAPGKGLEWVSAITWNSGHIDYADSVEGRFTISRDNAKNSLYLQMNSLRAEDTAVYYCAKVSYLSTASSLDYWGQGTLVTVSSGGGGSGGGGSGGGGSGGGGSDIQMTQSPSSLSASVGDRVTITCRASQGIRNYLAWYQQKPGKAPKLLIYAASTLQSGVPSRFSGSGSGTDFTLTISSLQPEDVATYYCQRYNRAPYTFGQGTKVEIK

SEQ ID NO: 74 - DNA, 2118 bp, Artificial Sequence
  I3F07-TNFai HC heavy chain
cagattcagctggctcagtctggcgccgaacttgtgaaacctggcgcctctgtgaagctgagctgcaaggccagcggcttcacctttcctgactactggatgcactgggtcaagcagaggcctggacagggactcgaatggatcggcgagatcgatcctcctaacggccggaccaactacaacgagaagttcaagagcaaggccacactgaccgtggacagcagcagcaataccgcctacatgcagctgagcagactgacctctgaggacagcgccgtgtactactgtgccagaggcatctactacgtggactactggggccagggcacaaccctgacagtttcttctgcttccaccaagggcccatccgtcttccccctggcgccctgctccaggagcacctccgagagcacagccgccctgggctgcctggtcaaggactacttccccgaaccggtgacggtgtcgtggaactcaggcgccctgaccagcggcgtgcacaccttcccggctgtcctacagtcctcaggactctactccctcagcagcgtggtgaccgtgccctccagcagcttgggcacgaagacctacacctgcaacgtagatcacaagcccagcaacaccaaggtggacaagagagttgagtccaaatatggtcccccatgcccaccatgcccagcacctgagttcctggggggaccatcagtcttcctgttccccccaaaacccaaggacactctcatgatctcccggacccctgaggtcacgtgcgtggtggtggacgtgagccaggaagaccccgaggtccagttcaactggtacgtggatggcgtggaggtgcataatgccaagacaaagccgcgggaggagcagttcaacagcacgtaccgtgtggtcagcgtcctcaccgtcctgcaccaggactggctgaacggcaaggagtacaagtgcaaggtctccaacaaaggcctcccgtcctccatcgagaaaaccatctccaaagccaaagggcagccccgagagccacaggtgtacaccctgcccccatcccaggaggagatgaccaagaaccaggtcagcctgacctgcctggtcaaaggcttctaccccagcgacatcgccgtggagtgggagagcaatgggcagccggagaacaactacaagaccacgcctcccgtgctggactccgacggctccttcttcctctacagcaggctaaccgtggacaagagcaggtggcaggaggggaatgtcttctcatgctccgtgatgcatgaggctctgcacaaccactacacacagaagagcctctccctgtctctgggtaaaggtggtggcggatctggcggcggaggaagcggaggcggaggatccgaagtgcaactggttgaatctggcggaggactggtgcagcctggaagaagcctgagactgtcttgtgccgccagcggcttcaccttcgatgattatgccatgcactgggtccgacaggcccctggaaaaggacttgaatgggtgtccgccatcacctggaacagcggccacatcgattacgccgatagcgtggaaggccggttcaccatcagcagagacaacgccaagaacagcctgtacctgcagatgaactccctgagagccgaggacaccgccgtgtactactgtgccaaagtgtcttacctgagcaccgcctccagcctggattattggggacagggcacactggtcacagtgtcctctggtggcggaggttctggcggaggtggtagtggtggcggtggaagtggtggcggcggatctgatatccagatgacacagagccctagcagcctgtctgcctctgtgggcgatagagtgaccatcacctgtagagccagccagggcatcagaaactacctggcctggtatcagcagaagcccggaaaggcccctaagctgctgatctatgccgcctctacactgcagagcggcgtgccatctagattttctggcagcggctctggcaccgacttcaccctgacaatttctagcctgcagcctgaggacgtggccacctactactgccagagatacaacagagccccttacaccttcggccagggcaccaaggtggaaatcaag

SEQ ID NO: 75 - protein, 482 aa, Artificial Sequence
  I3F07-TNFai LC light chain
DIVLTQSPLSLPVSLGDQASISCRSSQSLVHSNGNTYLHWYLQKPGQSPKLLIYKVSNRFSGVPDRFSGSGSGTDFTLKISRVEAEDLGVYFCSQSTHVPPTFGGGSKLEIKRTVAAPSVFIFPPSDEQLKSGTASVVCLLNNFYPREAKVQWKVDNALQSGNSQESVTEQDSKDSTYSLSSTLTLSKADYEKHKVYACEVTHQGLSSPVTKSFNRGECGGGGSGGGGSGGGGSEVQLVESGGGLVQPGRSLRLSCAASGFTFDDYAMHWVRQAPGKGLEWVSAITWNSGHIDYADSVEGRFTISRDNAKNSLYLQMNSLRAEDTAVYYCAKVSYLSTASSLDYWGQGTLVTVSSGGGGSGGGGSGGGGSGGGGSDIQMTQSPSSLSASVGDRVTITCRASQGIRNYLAWYQQKPGKAPKLLIYAASTLQSGVPSRFSGSGSGTDFTLTISSLQPEDVATYYCQRYNRAPYTFGQGTKVEIK

SEQ ID NO: 76 - DNA, 1446 bp, Artificial Sequence
  I3F07-TNFai LC light chain
gatatcgtgctgacacagagccctctgagcctgcctgtttctctgggagatcaggccagcatcagctgcagatcctctcagagcctggtgcacagcaacggcaatacctacctgcactggtatctgcagaagcccggccagtctcctaagctgctgatctacaaggtgtccaacaggttcagcggcgtgcccgatagattttctggctctggcagcggcaccgacttcaccctgaagatttctagagtggaagccgaggacctgggcgtgtacttctgttctcagtctacccacgtgccacctacctttggcggcggaagcaagctggaaatcaagcgtacggtggcggcgccatctgtcttcatcttcccgccatctgatgagcagttgaaatctggaactgcctctgttgtgtgcctgctgaataacttctatcccagagaggccaaagtacagtggaaggtggataacgccctccaatcgggtaactcccaggagagtgtcacagagcaggacagcaaggacagcacctacagcctcagcagcaccctgacgctgagcaaagcagactacgagaaacacaaagtctacgcctgcgaagtcacccatcagggcctgagctcgcccgtcacaaagagcttcaacaggggagagtgtggtggtggcggatctggcggcggaggaagcggaggcggaggatccgaagtgcaactggttgaatctggcggaggactggtgcagcctggaagaagcctgagactgtcttgtgccgccagcggcttcaccttcgatgattatgccatgcactgggtccgacaggcccctggaaaaggacttgaatgggtgtccgccatcacctggaacagcggccacatcgattacgccgatagcgtggaaggccggttcaccatcagcagagacaacgccaagaacagcctgtacctgcagatgaactccctgagagccgaggacaccgccgtgtactactgtgccaaagtgtcttacctgagcaccgcctccagcctggattattggggacagggcacactggtcacagtgtcctctggtggcggaggttctggcggaggtggtagtggtggcggtggaagtggtggcggcggatctgatatccagatgacacagagccctagcagcctgtctgcctctgtgggcgatagagtgaccatcacctgtagagccagccagggcatcagaaactacctggcctggtatcagcagaagcccggaaaggcccctaagctgctgatctatgccgcctctacactgcagagcggcgtgccatctagattttctggcagcggctctggcaccgacttcaccctgacaatttctagcctgcagcctgaggacgtggccacctactactgccagagatacaacagagccccttacaccttcggccagggcaccaaggtggaaatcaag

SEQ ID NO: 77 - protein, 711 aa, Artificial Sequence
  TNFai- I3F07 HC heavy chain
EVQLVESGGGLVQPGRSLRLSCAASGFTFDDYAMHWVRQAPGKGLEWVSAITWNSGHIDYADSVEGRFTISRDNAKNSLYLQMNSLRAEDTAVYYCAKVSYLSTASSLDYWGQGTLVTVSSASTKGPSVFPLAPCSRSTSESTAALGCLVKDYFPEPVTVSWNSGALTSGVHTFPAVLQSSGLYSLSSVVTVPSSSLGTKTYTCNVDHKPSNTKVDKRVESKYGPPCPPCPAPEFLGGPSVFLFPPKPKDTLMISRTPEVTCVVVDVSQEDPEVQFNWYVDGVEVHNAKTKPREEQFNSTYRVVSVLTVLHQDWLNGKEYKCKVSNKGLPSSIEKTISKAKGQPREPQVYTLPPSQEEMTKNQVSLTCLVKGFYPSDIAVEWESNGQPENNYKTTPPVLDSDGSFFLYSRLTVDKSRWQEGNVFSCSVMHEALHNHYTQKSLSLSLGKGGGGSGGGGSGGGGSQIQLAQSGAELVKPGASVKLSCKASGFTFPDYWMHWVKQRPGQGLEWIGEIDPPNGRTNYNEKFKSKATLTVDSSSNTAYMQLSRLTSEDSAVYYCARGIYYVDYWGQGTTLTVSSGGGGSGGGGSGGGGSGGGGSDIVLTQSPLSLPVSLGDQASISCRSSQSLVHSNGNTYLHWYLQKPGQSPKLLIYKVSNRFSGVPDRFSGSGSGTDFTLKISRVEAEDLGVYFCSQSTHVPPTFGGGSKLEIK

SEQ ID NO: 78 - DNA, 2133 bp, Artificial Sequence
  TNFai- I3F07 HC heavy chain
gaagtgcaactggttgaatctggcggaggactggtgcagcctggaagaagcctgagactgtcttgtgccgccagcggcttcaccttcgatgattatgccatgcactgggtccgacaggcccctggaaaaggacttgaatgggtgtccgccatcacctggaacagcggccacatcgattacgccgatagcgtggaaggccggttcaccatcagcagagacaacgccaagaacagcctgtacctgcagatgaactccctgagagccgaggacaccgccgtgtactactgtgccaaagtgtcttacctgagcaccgcctccagcctggattattggggacagggcacactggtcacagtgtcctctgcttccaccaagggcccatccgtcttccccctggcgccctgctccaggagcacctccgagagcacagccgccctgggctgcctggtcaaggactacttccccgaaccggtgacggtgtcgtggaactcaggcgccctgaccagcggcgtgcacaccttcccggctgtcctacagtcctcaggactctactccctcagcagcgtggtgaccgtgccctccagcagcttgggcacgaagacctacacctgcaacgtagatcacaagcccagcaacaccaaggtggacaagagagttgagtccaaatatggtcccccatgcccaccatgcccagcacctgagttcctggggggaccatcagtcttcctgttccccccaaaacccaaggacactctcatgatctcccggacccctgaggtcacgtgcgtggtggtggacgtgagccaggaagaccccgaggtccagttcaactggtacgtggatggcgtggaggtgcataatgccaagacaaagccgcgggaggagcagttcaacagcacgtaccgtgtggtcagcgtcctcaccgtcctgcaccaggactggctgaacggcaaggagtacaagtgcaaggtctccaacaaaggcctcccgtcctccatcgagaaaaccatctccaaagccaaagggcagccccgagagccacaggtgtacaccctgcccccatcccaggaggagatgaccaagaaccaggtcagcctgacctgcctggtcaaaggcttctaccccagcgacatcgccgtggagtgggagagcaatgggcagccggagaacaactacaagaccacgcctcccgtgctggactccgacggctccttcttcctctacagcaggctaaccgtggacaagagcaggtggcaggaggggaatgtcttctcatgctccgtgatgcatgaggctctgcacaaccactacacacagaagagcctctccctgtctctgggtaaaggtggtggcggatctggcggcggaggaagcggaggcggaggatcccagattcagctggctcagtctggcgccgaacttgtgaaacctggcgcctctgtgaagctgagctgcaaggccagcggcttcacctttcctgactactggatgcactgggtcaagcagaggcctggacagggactcgaatggatcggcgagatcgatcctcctaacggccggaccaactacaacgagaagttcaagagcaaggccacactgaccgtggacagcagcagcaataccgcctacatgcagctgagcagactgacctctgaggacagcgccgtgtactactgtgccagaggcatctactacgtggactactggggccagggcacaaccctgacagtttcttctggtggcggaggttctggcggaggtggtagtggtggcggtggaagtggtggcggcggatctgatatcgtgctgacacagagccctctgagcctgcctgtttctctgggagatcaggccagcatcagctgcagatcctctcagagcctggtgcacagcaacggcaatacctacctgcactggtatctgcagaagcccggccagtctcctaagctgctgatctacaaggtgtccaacaggttcagcggcgtgcccgatagattttctggctctggcagcggcaccgacttcaccctgaagatttctagagtggaagccgaggacctgggcgtgtacttctgttctcagtctacccacgtgccacctacctttggcggcggaagcaagctggaaatcaag

SEQ ID NO: 79 - protein, 477 aa, Artificial Sequence
  TNFai- I3F07 LC light chain
DIQMTQSPSSLSASVGDRVTITCRASQGIRNYLAWYQQKPGKAPKLLIYAASTLQSGVPSRFSGSGSGTDFTLTISSLQPEDVATYYCQRYNRAPYTFGQGTKVEIKRTVAAPSVFIFPPSDEQLKSGTASVVCLLNNFYPREAKVQWKVDNALQSGNSQESVTEQDSKDSTYSLSSTLTLSKADYEKHKVYACEVTHQGLSSPVTKSFNRGECGGGGSGGGGSGGGGSQIQLAQSGAELVKPGASVKLSCKASGFTFPDYWMHWVKQRPGQGLEWIGEIDPPNGRTNYNEKFKSKATLTVDSSSNTAYMQLSRLTSEDSAVYYCARGIYYVDYWGQGTTLTVSSGGGGSGGGGSGGGGSGGGGSDIVLTQSPLSLPVSLGDQASISCRSSQSLVHSNGNTYLHWYLQKPGQSPKLLIYKVSNRFSGVPDRFSGSGSGTDFTLKISRVEAEDLGVYFCSQSTHVPPTFGGGSKLEIK

SEQ ID NO: 80 - DNA, 1431 bp, Artificial Sequence
  TNFai- I3F07 LC light chain
gatatccagatgacacagagccctagcagcctgtctgcctctgtgggcgatagagtgaccatcacctgtagagccagccagggcatcagaaactacctggcctggtatcagcagaagcccggaaaggcccctaagctgctgatctatgccgcctctacactgcagagcggcgtgccatctagattttctggcagcggctctggcaccgacttcaccctgacaatttctagcctgcagcctgaggacgtggccacctactactgccagagatacaacagagccccttacaccttcggccagggcaccaaggtggaaatcaagcgtacggtggcggcgccatctgtcttcatcttcccgccatctgatgagcagttgaaatctggaactgcctctgttgtgtgcctgctgaataacttctatcccagagaggccaaagtacagtggaaggtggataacgccctccaatcgggtaactcccaggagagtgtcacagagcaggacagcaaggacagcacctacagcctcagcagcaccctgacgctgagcaaagcagactacgagaaacacaaagtctacgcctgcgaagtcacccatcagggcctgagctcgcccgtcacaaagagcttcaacaggggagagtgtggtggtggcggatctggcggcggaggaagcggaggcggaggatcccagattcagctggctcagtctggcgccgaacttgtgaaacctggcgcctctgtgaagctgagctgcaaggccagcggcttcacctttcctgactactggatgcactgggtcaagcagaggcctggacagggactcgaatggatcggcgagatcgatcctcctaacggccggaccaactacaacgagaagttcaagagcaaggccacactgaccgtggacagcagcagcaataccgcctacatgcagctgagcagactgacctctgaggacagcgccgtgtactactgtgccagaggcatctactacgtggactactggggccagggcacaaccctgacagtttcttctggtggcggaggttctggcggaggtggtagtggtggcggtggaagtggtggcggcggatctgatatcgtgctgacacagagccctctgagcctgcctgtttctctgggagatcaggccagcatcagctgcagatcctctcagagcctggtgcacagcaacggcaatacctacctgcactggtatctgcagaagcccggccagtctcctaagctgctgatctacaaggtgtccaacaggttcagcggcgtgcccgatagattttctggctctggcagcggcaccgacttcaccctgaagatttctagagtggaagccgaggacctgggcgtgtacttctgttctcagtctacccacgtgccacctacctttggcggcggaagcaagctggaaatcaag

SEQ ID NO: 81 - protein, 447 aa, Artificial Sequence
  Ref. Ab heavy chain
EVQLLESGGGLVQPGGSLRLSCAASGFTFNSYAMSWVRQAPGKGLEWVSIISGSGGFTYYADSVKGRFTISRDNSRTTLYLQMNSLRAEDTAVYYCAKDRLVAPGTFDYWGQGALVTVSSASTKGPSVFPLAPCSRSTSESTAALGCLVKDYFPEPVTVSWNSGALTSGVHTFPAVLQSSGLYSLSSVVTVPSSSLGTKTYTCNVDHKPSNTKVDKRVESKYGPPCPPCPAPEFLGGPSVFLFPPKPKDTLMISRTPEVTCVVVDVSQEDPEVQFNWYVDGVEVHNAKTKPREEQFNSTYRVVSVLTVLHQDWLNGKEYKCKVSNKGLPSSIEKTISKAKGQPREPQVYTLPPSQEEMTKNQVSLTCLVKGFYPSDIAVEWESNGQPENNYKTTPPVLDSDGSFFLYSRLTVDKSRWQEGNVFSCSVMHEALHNHYTQKSLSLSLGK

SEQ ID NO: 82 - protein, 214 aa, Artificial Sequence
  Ref. Ab light chain
DIQMTQSPSSLSASVGDRVTITCRASQGISSWLAWYQQKPEKAPKSLIYAASSLQSGVPSRFSGSGSGTDFTLTISSLQPEDFATYYCQQYNSYPYTFGQGTKLEIKRTVAAPSVFIFPPSDEQLKSGTASVVCLLNNFYPREAKVQWKVDNALQSGNSQESVTEQDSKDSTYSLSSTLTLSKADYEKHKVYACEVTHQGLSSPVTKSFNRGEC

SEQ ID NO: 83 - protein, 448 aa, Artificial Sequence
  Ref. TNFai heavy chain
EVQLVESGGGLVQPGRSLRLSCAASGFTFDDYAMHWVRQAPGKGLEWVSAITWNSGHIDYADSVEGRFTISRDNAKNSLYLQMNSLRAEDTAVYYCAKVSYLSTASSLDYWGQGTLVTVSSASTKGPSVFPLAPCSRSTSESTAALGCLVKDYFPEPVTVSWNSGALTSGVHTFPAVLQSSGLYSLSSVVTVPSSSLGTKTYTCNVDHKPSNTKVDKRVESKYGPPCPPCPAPEFLGGPSVFLFPPKPKDTLMISRTPEVTCVVVDVSQEDPEVQFNWYVDGVEVHNAKTKPREEQFNSTYRVVSVLTVLHQDWLNGKEYKCKVSNKGLPSSIEKTISKAKGQPREPQVYTLPPSQEEMTKNQVSLTCLVKGFYPSDIAVEWESNGQPENNYKTTPPVLDSDGSFFLYSRLTVDKSRWQEGNVFSCSVMHEALHNHYTQKSLSLSLGK

SEQ ID NO: 84 - protein, 214 aa, Artificial Sequence
  Ref. TNFai light chain
DIQMTQSPSSLSASVGDRVTITCRASQGIRNYLAWYQQKPGKAPKLLIYAASTLQSGVPSRFSGSGSGTDFTLTISSLQPEDVATYYCQRYNRAPYTFGQGTKVEIKRTVAAPSVFIFPPSDEQLKSGTASVVCLLNNFYPREAKVQWKVDNALQSGNSQESVTEQDSKDSTYSLSSTLTLSKADYEKHKVYACEVTHQGLSSPVTKSFNRGEC

SEQ ID NO: 85 - protein, 710 aa, Artificial Sequence
  O4L-TNFai HC heavy chain
EVQLLESGGGLVQPGGSLRLSCAASGFTFNSYAMSWVRQAPGKGLEWVSIISGSGGFTYYADSVKGRFTISRDNSRTTLYLQMNSLRAEDTAVYYCAKDRLVAPGTFDYWGQGALVTVSSASTKGPSVFPLAPCSRSTSESTAALGCLVKDYFPEPVTVSWNSGALTSGVHTFPAVLQSSGLYSLSSVVTVPSSSLGTKTYTCNVDHKPSNTKVDKRVESKYGPPCPPCPAPEFLGGPSVFLFPPKPKDTLMISRTPEVTCVVVDVSQEDPEVQFNWYVDGVEVHNAKTKPREEQFNSTYRVVSVLTVLHQDWLNGKEYKCKVSNKGLPSSIEKTISKAKGQPREPQVYTLPPSQEEMTKNQVSLTCLVKGFYPSDIAVEWESNGQPENNYKTTPPVLDSDGSFFLYSRLTVDKSRWQEGNVFSCSVMHEALHNHYTQKSLSLSLGKGGGGSGGGGSGGGGSEVQLVESGGGLVQPGRSLRLSCAASGFTFDDYAMHWVRQAPGKGLEWVSAITWNSGHIDYADSVEGRFTISRDNAKNSLYLQMNSLRAEDTAVYYCAKVSYLSTASSLDYWGQGTLVTVSSGGGGSGGGGSGGGGSGGGGSDIQMTQSPSSLSASVGDRVTITCRASQGIRNYLAWYQQKPGKAPKLLIYAASTLQSGVPSRFSGSGSGTDFTLTISSLQPEDVATYYCQRYNRAPYTFGQGTKVEIK

SEQ ID NO: 86 - DNA, 2130 bp, Artificial Sequence
  O4L-TNFai HC heavy chain
gaggtgcagctgctggaaagcggcggaggactggtgcagcctggcggcagcctgagactgtcttgcgccgccagcggcttcaccttcaacagctacgccatgagctgggtccgacaggcccctggcaagggcctggaatgggtgtccatcatcagcggcagcggcggctttacctactacgccgacagcgtgaagggccggttcaccatcagccgggacaacagccggaccaccctgtacctgcagatgaacagcctgcgggccgaggacaccgccgtgtactactgcgccaaggacagactggtggccccaggcaccttcgactattggggacagggcgccctcgtgaccgtgtcctctgcttccaccaagggcccatccgtcttccccctggcgccctgctccaggagcacctccgagagcacagccgccctgggctgcctggtcaaggactacttccccgaaccggtgacggtgtcgtggaactcaggcgccctgaccagcggcgtgcacaccttcccggctgtcctacagtcctcaggactctactccctcagcagcgtggtgaccgtgccctccagcagcttgggcacgaagacctacacctgcaacgtagatcacaagcccagcaacaccaaggtggacaagagagttgagtccaaatatggtcccccatgcccaccatgcccagcacctgagttcctggggggaccatcagtcttcctgttccccccaaaacccaaggacactctcatgatctcccggacccctgaggtcacgtgcgtggtggtggacgtgagccaggaagaccccgaggtccagttcaactggtacgtggatggcgtggaggtgcataatgccaagacaaagccgcgggaggagcagttcaacagcacgtaccgtgtggtcagcgtcctcaccgtcctgcaccaggactggctgaacggcaaggagtacaagtgcaaggtctccaacaaaggcctcccgtcctccatcgagaaaaccatctccaaagccaaagggcagccccgagagccacaggtgtacaccctgcccccatcccaggaggagatgaccaagaaccaggtcagcctgacctgcctggtcaaaggcttctaccccagcgacatcgccgtggagtgggagagcaatgggcagccggagaacaactacaagaccacgcctcccgtgctggactccgacggctccttcttcctctacagcaggctaaccgtggacaagagcaggtggcaggaggggaatgtcttctcatgctccgtgatgcatgaggctctgcacaaccactacacacagaagagcctctccctgtctctgggtaaaggtggtggcggatctggcggcggaggaagcggaggcggaggatccgaagtgcaactggttgaatctggcggaggactggtgcagcctggaagaagcctgagactgtcttgtgccgccagcggcttcaccttcgatgattatgccatgcactgggtccgacaggcccctggaaaaggacttgaatgggtgtccgccatcacctggaacagcggccacatcgattacgccgatagcgtggaaggccggttcaccatcagcagagacaacgccaagaacagcctgtacctgcagatgaactccctgagagccgaggacaccgccgtgtactactgtgccaaagtgtcttacctgagcaccgcctccagcctggattattggggacagggcacactggtcacagtgtcctctggtggcggaggttctggcggaggtggtagtggtggcggtggaagtggtggcggcggatctgatatccagatgacacagagccctagcagcctgtctgcctctgtgggcgatagagtgaccatcacctgtagagccagccagggcatcagaaactacctggcctggtatcagcagaagcccggaaaggcccctaagctgctgatctatgccgcctctacactgcagagcggcgtgccatctagattttctggcagcggctctggcaccgacttcaccctgacaatttctagcctgcagcctgaggacgtggccacctactactgccagagatacaacagagccccttacaccttcggccagggcaccaaggtggaaatcaag

SEQ ID NO: 87 - protein, 477 aa, Artificial Sequence
  O4L-TNFai LC light chain
DIQMTQSPSSLSASVGDRVTITCRASQGISSWLAWYQQKPEKAPKSLIYAASSLQSGVPSRFSGSGSGTDFTLTISSLQPEDFATYYCQQYNSYPYTFGQGTKLEIKRTVAAPSVFIFPPSDEQLKSGTASVVCLLNNFYPREAKVQWKVDNALQSGNSQESVTEQDSKDSTYSLSSTLTLSKADYEKHKVYACEVTHQGLSSPVTKSFNRGECGGGGSGGGGSGGGGSEVQLVESGGGLVQPGRSLRLSCAASGFTFDDYAMHWVRQAPGKGLEWVSAITWNSGHIDYADSVEGRFTISRDNAKNSLYLQMNSLRAEDTAVYYCAKVSYLSTASSLDYWGQGTLVTVSSGGGGSGGGGSGGGGSGGGGSDIQMTQSPSSLSASVGDRVTITCRASQGIRNYLAWYQQKPGKAPKLLIYAASTLQSGVPSRFSGSGSGTDFTLTISSLQPEDVATYYCQRYNRAPYTFGQGTKVEIK

SEQ ID NO: 88 - DNA, 1431 bp, Artificial Sequence
  O4L-TNFai LC light chain
gacatccagatgacccagagccccagcagcctgagcgccagcgtgggcgacagagtgaccatcacctgtcgggccagccagggcatcagcagctggctggcctggtatcagcagaagcccgagaaggcccccaagagcctgatctacgccgccagctctctgcagagcggcgtgcccagcagattcagcggcagcggctccggcaccgacttcaccctgaccatcagcagcctgcagcccgaggacttcgccacctactactgccagcagtacaacagctacccctacaccttcggccagggcaccaagctggaaatcaagcgtacggtggcggcgccatctgtcttcatcttcccgccatctgatgagcagttgaaatctggaactgcctctgttgtgtgcctgctgaataacttctatcccagagaggccaaagtacagtggaaggtggataacgccctccaatcgggtaactcccaggagagtgtcacagagcaggacagcaaggacagcacctacagcctcagcagcaccctgacgctgagcaaagcagactacgagaaacacaaagtctacgcctgcgaagtcacccatcagggcctgagctcgcccgtcacaaagagcttcaacaggggagagtgtggtggtggcggatctggcggcggaggaagcggaggcggaggatccgaagtgcaactggttgaatctggcggaggactggtgcagcctggaagaagcctgagactgtcttgtgccgccagcggcttcaccttcgatgattatgccatgcactgggtccgacaggcccctggaaaaggacttgaatgggtgtccgccatcacctggaacagcggccacatcgattacgccgatagcgtggaaggccggttcaccatcagcagagacaacgccaagaacagcctgtacctgcagatgaactccctgagagccgaggacaccgccgtgtactactgtgccaaagtgtcttacctgagcaccgcctccagcctggattattggggacagggcacactggtcacagtgtcctctggtggcggaggttctggcggaggtggtagtggtggcggtggaagtggtggcggcggatctgatatccagatgacacagagccctagcagcctgtctgcctctgtgggcgatagagtgaccatcacctgtagagccagccagggcatcagaaactacctggcctggtatcagcagaagcccggaaaggcccctaagctgctgatctatgccgcctctacactgcagagcggcgtgccatctagattttctggcagcggctctggcaccgacttcaccctgacaatttctagcctgcagcctgaggacgtggccacctactactgccagagatacaacagagccccttacaccttcggccagggcaccaaggtggaaatcaag

SEQ ID NO: 89 - protein, 5 aa, Artificial Sequence
  Humira VH CDR 1
DYAMH

SEQ ID NO: 90 - protein, 17 aa, Artificial Sequence
  Humira VH CDR 2
AITWNSGHIDYADSVEG

SEQ ID NO: 91 - protein, 12 aa, Artificial Sequence
  Humira VH CDR 3
VSYLSTASSLDY

SEQ ID NO: 92 - protein, 11 aa, Artificial Sequence
  Humira VL CDR 1
RASQGIRNYLA

SEQ ID NO: 93 - protein, 7 aa, Artificial Sequence
  Humira VL CDR 2
AASTLQS

SEQ ID NO: 94 - protein, 9 aa, Artificial Sequence
  Humira VL CDR 3
QRYNRAPYT